European Patent Specification EP 3 811 973 B1, published November 27, 2024. Title: A Composition for Preventing or Treating A Neurodegenerative Disease. Applicant: KYOTO UNIVERSITY. The sequence listing filed with the application follows.

SEQUENCE LISTING (38 sequences)

SEQ ID NO: 1 - RNA, 21 nt, Homo sapiens
gugcauuguaguugcauugca

SEQ ID NO: 2 - DNA, 23 bp, Artificial
  DNA encoding CRISPR guide RNA
gctgcccgccaggaggtatgcgg

SEQ ID NO: 3 - DNA, 23 bp, Artificial
  DNA encoding CRISPR guide RNA
tgtagttgcattgcatgttctgg

SEQ ID NO: 4 - DNA, 20 bp, Artificial
  DNA encoding CRISPR guide RNA
tgcaacagcaatgcaccgcg

SEQ ID NO: 5 - DNA, 20 bp, Artificial
  DNA encoding CRISPR guide RNA
tcggcagtgcagcccggagc

SEQ ID NO: 6 - DNA, 22 bp, Artificial
  Primer
aacagtcccactggtcgtagat

SEQ ID NO: 7 - DNA, 22 bp, Artificial
  Primer
tgttgcagaaagcgaatgtagt

SEQ ID NO: 8 - DNA, 18 bp, Artificial
  Primer
aggagaacatggtgctga

SEQ ID NO: 9 - DNA, 18 bp, Artificial
  Primer
taaaggagaggcacagga

SEQ ID NO: 10 - DNA, 20 bp, Artificial
  Primer
agctggtcaagacttggcaa

SEQ ID NO: 11 - DNA, 20 bp, Artificial
  Primer
aggttgcattcgattctgca

SEQ ID NO: 12 - DNA, 23 bp, Artificial
  Primer
gtcctctttcccgcattatctgg

SEQ ID NO: 13 - DNA, 23 bp, Artificial
  Primer
agttcctggaaggtcttgttcac

SEQ ID NO: 14 - DNA, 20 bp, Artificial
  Primer
agaaacggctaccacatcca

SEQ ID NO: 15 - DNA, 20 bp, Artificial
  Primer
ccctccaatggatcctcgtt

SEQ ID NO: 16 - DNA, 20 bp, Artificial
  Primer
gtggagcagtctcaacgtca

SEQ ID NO: 17 - DNA, 20 bp, Artificial
  Primer
tggtaggtctcacccaggag

SEQ ID NO: 18 - DNA, 20 bp, Artificial
  Primer
cgggccaaggtgaacagtat

SEQ ID NO: 19 - DNA, 20 bp, Artificial
  Primer
gatgtccattgcggcatgtc

SEQ ID NO: 20 - DNA, 20 bp, Artificial
  Primer
cgcggttctattttgttggt

SEQ ID NO: 21 - DNA, 20 bp, Artificial
  Primer
agtcggcatcgtttatggtc

SEQ ID NO: 22 - DNA, 50 bp, Homo sapiens
acagacttaaacaaaatatacaatgcaaatgtaattttttgttgtttaag

SEQ ID NO: 23 - DNA, 50 bp, Artificial
  Mutant of SPAST 3'UTR fragment
acagacttaaacaaaatatacccgtaaaatgtaattttttgttgtttaag

SEQ ID NO: 24 - DNA, 12 bp, Artificial
  Synthetic
  misc_feature (1)..(1), (5)..(5), (7)..(7), (9)..(9): LNA
  misc_feature (3)..(3), (11)..(11): 5-methylcytosine LNA
aactacaatgca

SEQ ID NO: 25 - DNA, 12 bp, Artificial
  Synthetic
  misc_feature (1)..(1), (5)..(5), (7)..(7), (9)..(9): LNA
  misc_feature (3)..(3), (11)..(11): 5-methylcytosine LNA
aacaatactacg

SEQ ID NO: 26 - DNA, 114 bp, Artificial
  premiR-33a without seed sequence
ctgtggcgcaacgcaattagtgataacttcgtatagcatacattatacgaagttatgtttgttaccatttgtgttctaatggtacccatgcaatgtttccacagtgcatcacag

SEQ ID NO: 27 - DNA, 87 bp, Artificial
  premiR-33b without seed sequence
gcgggcgggcgcaacgcaattagtgataacttcgtatagcatacattatacgaagttatgtttgttaccatttgcccctggcaccac

SEQ ID NO: 28 - DNA, 24 bp, Homo sapiens
tgccctcaaccacgtggtccagct

SEQ ID NO: 29 - DNA, 25 bp, Homo sapiens
tccattgacaaggccgtgcagctgt

SEQ ID NO: 30 - RNA, 39 nt, Homo sapiens
aaaacagacuuaaacaaaauauacaaugcaaauguaauu

SEQ ID NO: 31 - RNA, 39 nt, Pan troglodytes
aaaacaaacuuaaacaaaauauacaaugcaaauggaauu

SEQ ID NO: 32 - RNA, 39 nt, Macaca mulatta
aaaacaaacuuaaacaaaauauacaaugcaaauagaauu

SEQ ID NO: 33 - RNA, 39 nt, Canis lupus familiaris
aaaacaaauuuaaauaaaauauacaaugcaaauggagua

SEQ ID NO: 34 - RNA, 39 nt, Bos taurus
aaaauaaauuuaaauaaaguauacaaugcaaauggaaua

SEQ ID NO: 35 - RNA, 37 nt, Mus musculus
aagacagaccuaaauaaaauaugcaauaugaauggaa

SEQ ID NO: 36 - DNA, 40 bp, Homo sapiens
tttaacttcaaaatacgtgagtgctctgtttccaatattg

SEQ ID NO: 37 - DNA, 40 bp, Homo sapiens
tttaacttcaaaatacatgagtgctctgtttccaatattg

SEQ ID NO: 38 - DNA, 31 bp, Homo sapiens
ctccttctcccaccagcattgtcttcccatt